European Patent Specification EP 3 755 815 B1, published July 12, 2023. Title: Biomarker zur Feststellung einer möglichen Unverträglichkeit gegenüber Metallimplantaten. Applicant: Klinikum der Universität München. The sequence listing filed with the application follows.

SEQUENCE LISTING (13 sequences)

SEQ ID NO: 1 - DNA, 51 bp, Homo sapiens
  rs1143627
agcctcctacttctgcttttgaaagcyataaaaacagcgagggagaactgg

SEQ ID NO: 2 - DNA, 86 bp, Homo sapiens
  rs2234663 repeat
atcctggggaaagtgagggaaatatggacatcacatggaacaacatccaggagactcaggcctctaggagtaactgggtagtgtgc

SEQ ID NO: 3 - DNA, 52 bp, Homo sapiens
  rs1143634
ctccacatttcagaacctatcttcttygacacatgggataacgaggcttatg

SEQ ID NO: 4 - DNA, 52 bp, Homo sapiens
  rs16944
ctaccttgggtgctgttctctgcctcrggagctctctgtcaattgcaggagc

SEQ ID NO: 5 - DNA, 205 bp, Homo sapiens
  rs2234663 two repeats
actcctattgacctggagcacaggtatcctggggaaagtgagggaaatatggacatcacatggaacaacatccaggagactcaggcctctaggagtaactgggtagtgtgcatcctggggaaagtgagggaaatatggacatcacatggaacaacatccaggagactcaggcctctaggagtaactgggtagtgtgcttggttta

SEQ ID NO: 6 - DNA, 291 bp, Homo sapiens
  rs2234663 three repeats
actcctattgacctggagcacaggtatcctggggaaagtgagggaaatatggacatcacatggaacaacatccaggagactcaggcctctaggagtaactgggtagtgtgcatcctggggaaagtgagggaaatatggacatcacatggaacaacatccaggagactcaggcctctaggagtaactgggtagtgtgcatcctggggaaagtgagggaaatatggacatcacatggaacaacatccaggagactcaggcctctaggagtaactgggtagtgtgcttggttta

SEQ ID NO: 7 - DNA, 377 bp, Homo sapiens
  rs2234663 four repeats
actcctattgacctggagcacaggtatcctggggaaagtgagggaaatatggacatcacatggaacaacatccaggagactcaggcctctaggagtaactgggtagtgtgcatcctggggaaagtgagggaaatatggacatcacatggaacaacatccaggagactcaggcctctaggagtaactgggtagtgtgcatcctggggaaagtgagggaaatatggacatcacatggaacaacatccaggagactcaggcctctaggagtaactgggtagtgtgcatcctggggaaagtgagggaaatatggacatcacatggaacaacatccaggagactcaggcctctaggagtaactgggtagtgtgcttggttta

SEQ ID NO: 8 - DNA, 463 bp, Homo sapiens
  rs2234663 five repeats
actcctattgacctggagcacaggtatcctggggaaagtgagggaaatatggacatcacatggaacaacatccaggagactcaggcctctaggagtaactgggtagtgtgcatcctggggaaagtgagggaaatatggacatcacatggaacaacatccaggagactcaggcctctaggagtaactgggtagtgtgcatcctggggaaagtgagggaaatatggacatcacatggaacaacatccaggagactcaggcctctaggagtaactgggtagtgtgcatcctggggaaagtgagggaaatatggacatcacatggaacaacatccaggagactcaggcctctaggagtaactgggtagtgtgcatcctggggaaagtgagggaaatatggacatcacatggaacaacatccaggagactcaggcctctaggagtaactgggtagtgtgcttggttta

SEQ ID NO: 9 - DNA, 549 bp, Homo sapiens
  rs2234663 six repeats
actcctattgacctggagcacaggtatcctggggaaagtgagggaaatatggacatcacatggaacaacatccaggagactcaggcctctaggagtaactgggtagtgtgcatcctggggaaagtgagggaaatatggacatcacatggaacaacatccaggagactcaggcctctaggagtaactgggtagtgtgcatcctggggaaagtgagggaaatatggacatcacatggaacaacatccaggagactcaggcctctaggagtaactgggtagtgtgcatcctggggaaagtgagggaaatatggacatcacatggaacaacatccaggagactcaggcctctaggagtaactgggtagtgtgcatcctggggaaagtgagggaaatatggacatcacatggaacaacatccaggagactcaggcctctaggagtaactgggtagtgtgcatcctggggaaagtgagggaaatatggacatcacatggaacaacatccaggagactcaggcctctaggagtaactgggtagtgtgcttggttta

SEQ ID NO: 10 - DNA, 22 bp, Artificial Sequence
  Primer
tcttttcccctttcctttaact

SEQ ID NO: 11 - DNA, 23 bp, Artificial Sequence
  Primer
gagagactcccttagcacctagt

SEQ ID NO: 12 - DNA, 17 bp, Artificial Sequence
  Primer
cccctcagcaacactcc

SEQ ID NO: 13 - DNA, 17 bp, Artificial Sequence
  Primer
ggtcagaagggcagaga